European Patent Application EP 4 442 704 A1, published October 9, 2024. Title: Peptide having framework sequences for implementing random sequences and peptide library comprising thereof. Applicant: 株式会社Ｅｐｓｉｌｏｎ　Ｍｏｌｅｃｕｌａｒ　Ｅｎｇｉｎｅｅｒｉｎｇ. Application WO, filed November 30, 2022. The sequence listing filed with the application follows.

SEQUENCE LISTING (37 sequences)

SEQ ID NO: 1 - protein, 25 aa, synthetic construct [sequence omitted]

SEQ ID NO: 2 - protein, 14 aa, synthetic construct
  VARIANT 2: note = X can be any amino acid
  VARIANT 10: note = X can be any amino acid
WXRQAPGKGXEXVA

SEQ ID NO: 3 - protein, 14 aa, synthetic construct
WYRQAPGKGLEWVA

SEQ ID NO: 4 - protein, 14 aa, synthetic construct
WVRQAPGKGLEWVA

SEQ ID NO: 5 - protein, 14 aa, synthetic construct
WFRQAPGKGREFVA

SEQ ID NO: 6 - protein, 14 aa, synthetic construct
WFRQAPGKGREGVA

SEQ ID NO: 7 - protein, 32 aa, synthetic construct
  VARIANT 13: note = X can be any amino acid
  VARIANT 31: note = X can be any amino acid
  VARIANT 32: note = X can be any amino acid
RFTISRDNAKNTXYLQMNSLRAEDTAVYYCXX

SEQ ID NO: 8 - protein, 32 aa, synthetic construct
RFTISRDNAKNTLYLQMNSLRAEDTAVYYCNA

SEQ ID NO: 9 - protein, 32 aa, synthetic construct
RFTISRDNAKNTLYLQMNSLRAEDTAVYYCNV

SEQ ID NO: 10 - protein, 32 aa, synthetic construct
RFTISRDNAKNTLYLQMNSLRAEDTAVYYCNR

SEQ ID NO: 11 - protein, 32 aa, synthetic construct
RFTISRDNAKNTLYLQMNSLRAEDTAVYYCNL

SEQ ID NO: 12 - protein, 9 aa, synthetic construct
FRUPRIGHT

SEQ ID NO: 13 - protein, 32 aa, synthetic construct
RFTISRDNAKNTVYLQMNSLRAEDTAVYYCNV

SEQ ID NO: 14 - protein, 32 aa, synthetic construct
RFTISRDNAKNTVYLQMNSLRAEDTAVYYCNR

SEQ ID NO: 15 - protein, 32 aa, synthetic construct
RFTISRDNAKNTVYLQMNSLRAEDTAVYYCNL

SEQ ID NO: 16 - protein, 32 aa, synthetic construct
RFTISRDNAKNTLYLQMNSLRAEDTAVYYCAV

SEQ ID NO: 17 - protein, 32 aa, synthetic construct
RFTISRDNAKNTLYLQMNSLRAEDTAVYYCAR

SEQ ID NO: 18 - protein, 32 aa, synthetic construct
RFTISRDNAKNTLYLQMNSLRAEDTAVYYCAL

SEQ ID NO: 19 - protein, 32 aa, synthetic construct
RFTISRDNAKNTVYLQMNSLRAEDTAVYYCAV

SEQ ID NO: 20 - protein, 32 aa, synthetic construct
RFTISRDNAKNTVYLQMNSLRAEDTAVYYCAR

SEQ ID NO: 21 - protein, 32 aa, synthetic construct
RFTISRDNAKNTVYLQMNSLRAEDTAVYYCAL

SEQ ID NO: 22 - protein, 32 aa, synthetic construct
RFTISRDNAKNTLYLQMNSLRAEDTAVYYCKA

SEQ ID NO: 23 - protein, 32 aa, synthetic construct
RFTISRDNAKNTLYLQMNSLRAEDTAVYYCKV

SEQ ID NO: 24 - protein, 32 aa, synthetic construct
RFTISRDNAKNTLYLQMNSLRAEDTAVYYCKR

SEQ ID NO: 25 - protein, 32 aa, synthetic construct
RFTISRDNAKNTLYLQMNSLRAEDTAVYYCKL

SEQ ID NO: 26 - protein, 32 aa, synthetic construct
RFTISRDNAKNTVYLQMNSLRAEDTAVYYCKA

SEQ ID NO: 27 - protein, 32 aa, synthetic construct
RFTISRDNAKNTVYLQMNSLRAEDTAVYYCKV

SEQ ID NO: 28 - protein, 32 aa, synthetic construct
RFTISRDNAKNTVYLQMNSLRAEDTAVYYCKR

SEQ ID NO: 29 - protein, 32 aa, synthetic construct
RFTISRDNAKNTVYLQMNSLRAEDTAVYYCKL

SEQ ID NO: 30 - protein, 32 aa, synthetic construct
RFTISRDNAKNTLYLQMNSLRAEDTAVYYCAA

SEQ ID NO: 31 - protein, 32 aa, synthetic construct
RFTISRDNAKNTVYLQMNSLRAEDTAVYYCAA

SEQ ID NO: 32 - protein, 11 aa, synthetic construct
WGQGTLVTVSS

SEQ ID NO: 33 - DNA, 23 bp, synthetic construct
  source 1..23: mol_type = other DNA
  misc_feature 3: note = n is guanosine
  misc_feature 12: note = n is 3-cyanovinylcarbazole
aanaatttccangccgccccccg

SEQ ID NO: 34 - protein, 25 aa, synthetic construct
EVQLLESGGGLVQPGGSLRLSCAAS

SEQ ID NO: 35 - protein, 14 aa, synthetic construct
WVRQAPGKGLEWVS

SEQ ID NO: 36 - protein, 32 aa, synthetic construct
RFTISRDNSKNTLYLQMNSLRAEDTAVYYCAK

SEQ ID NO: 37 - protein, 11 aa, synthetic construct
WGQGTLVTVSS